European Patent Specification EP 3 805 409 B1, published May 15, 2024. Title: Quantitative PCR Probe. Applicant: Takeda Pharmaceutical Company Limited. The sequence listing filed with the application follows.

SEQUENCE LISTING (8 sequences)

SEQ ID NO: 1 - DNA, 508 bp, Homo sapiens
  Target range for qPCR probe on human LINE-1 gene (antisense strand)
ccattactgggtatatacccaaatgagtataaatcatgctgctataaagacacatgcacacgtatgtttattgcggcactattcacaatagcaaagacttggaaccaacccaaatgtccaacaatgatagactggattaagaaaatgtggcacatatacaccatggaatactatgcagccataaaaaatgatgagttcatatcctttgtagggacatggatgaaattggaaaccatcattctcagtaaactatcgcaagaacaaaaaaccaaacaccgcatattctcactcataggtgggaattgaacaatgagatcacatggacacaggaaggggaatatcacactctggggactgtggtggggttgggggaggggggagggatagtattgggagatatacctaatgctagatgacacattagtgggtgcagcgcaccagcatggcacatgtatacatatgtaactaacctgcacaatgtgcacatgtaccctaaaacttagagtat

SEQ ID NO: 2 - DNA, 508 bp, Homo sapiens
  Target range for qPCR probe on human LINE-1 gene (sense strand)
atactctaagttttagggtacatgtgcacattgtgcaggttagttacatatgtatacatgtgccatgctggtgcgctgcacccactaatgtgtcatctagcattaggtatatctcccaatactatccctcccccctcccccaaccccaccacagtccccagagtgtgatattccccttcctgtgtccatgtgatctcattgttcaattcccacctatgagtgagaatatgcggtgtttggttttttgttcttgcgatagtttactgagaatgatggtttccaatttcatccatgtccctacaaaggatatgaactcatcattttttatggctgcatagtattccatggtgtatatgtgccacattttcttaatccagtctatcattgttggacatttgggttggttccaagtctttgctattgtgaatagtgccgcaataaacatacgtgtgcatgtgtctttatagcagcatgatttatactcatttgggtatatacccagtaatgg

SEQ ID NO: 3 - DNA, 21 bp, Artificial Sequence
  qPCR Probe for human LINE-1 gene of Examples 1 and 2
cactaatgtgtcatctagcat

SEQ ID NO: 4 - DNA, 18 bp, Artificial Sequence
  qPCR Forward Primer for human LINE-1 gene of Examples 1 and 2
catgtgccatgctggtgc

SEQ ID NO: 5 - DNA, 27 bp, Artificial Sequence
  qPCR Reverse Primer for human LINE-1 gene of Examples 1 and 2
ccattactgggtatatacccaaatgag

SEQ ID NO: 6 - DNA, 23 bp, Artificial Sequence
  qPCR Probe for human LINE-1 gene of Example 3
tgagttcatatcctttgtaggga

SEQ ID NO: 7 - DNA, 27 bp, Artificial Sequence
  qPCR Reverse Primer for human LINE-1 gene of Example 3
ccattactgggtatatacccaaatgag

SEQ ID NO: 8 - DNA, 19 bp, Artificial Sequence
  qPCR Forward Primer for human LINE-1 gene of Example 3
gcgctgcacccactaatgt